European Patent Specification EP 4 073 097 B1, published July 3, 2024. Title: NOVEL INSULIN ANALOGUES AND USES THEREOF. Applicant: Novo Nordisk A/S. The sequence listing filed with the application follows.

SEQUENCE LISTING (9 sequences)

SEQ ID NO: 1 - protein, 21 aa, Homo sapiens
GIVEQCCTSICSLYQLENYCN

SEQ ID NO: 2 - protein, 30 aa, Homo sapiens
FVNQHLCGSHLVEALYLVCGERGFFYTPKT

SEQ ID NO: 3 - protein, 21 aa, Artificial Sequence
  A chain of analogue [A9E] of human insulin of Example 1, 2, 3 and 4
GIVEQCCTEICSLYQLENYCN

SEQ ID NO: 4 - protein, 29 aa, Artificial Sequence
  B-chain analogue [B3E, B26E, desB30] of human insulin of example 1
FVEQHLCGSHLVEALYLVCGERGFFETPK

SEQ ID NO: 5 - protein, 29 aa, Artificial Sequence
  B-chain analogue [B3E, B27E, B28E, desB30] of human insulin of example 2
FVEQHLCGSHLVEALYLVCGERGFFYEEK

SEQ ID NO: 6 - protein, 30 aa, Artificial Sequence
  B-chain analogue [B3E, B26E] of human insulin of example 3
FVEQHLCGSHLVEALYLVCGERGFFETPKT

SEQ ID NO: 7 - protein, 30 aa, Artificial Sequence
  B-chain analogue [B3E, B27E, B28E] of human insulin of example 4
FVEQHLCGSHLVEALYLVCGERGFFYEEKT

SEQ ID NO: 8 - protein, 21 aa, Artificial Sequence
  A chain of analogue [A9D] of human insulin of Example 5
GIVEQCCTDICSLYQLENYCN

SEQ ID NO: 9 - protein, 21 aa, Artificial Sequence
  A chain of analogue [A9E, A21A] of human insulin of Example 6
GIVEQCCTEICSLYQLENYCA